European Patent Application EP 4 420 672 A1, published August 28, 2024. Title: 寡肽在治疗牙龈发炎和牙龈萎缩及修复口腔黏膜中的用途. Applicant: 庄国昇. Application WO PCT/CN2022/125610, filed October 17, 2022. The sequence listing filed with the application follows.

SEQUENCE LISTING (4 sequences)

SEQ ID NO: 1 - protein, 4 aa, artificial sequence
GEKG

SEQ ID NO: 2 - protein, 5 aa, artificial sequence
GEKGF

SEQ ID NO: 3 - protein, 5 aa, artificial sequence
KTTKS

SEQ ID NO: 4 - protein, 6 aa, artificial sequence
KTTKSF